European Patent Specification EP 3 427 061 B1, published December 6, 2023. Title: IN VITRO METHOD FOR IDENTIFYING THORACIC AORTIC ANEURYSM (TAA) IN A SUBJECT. Applicant: CNIC Fundación Centro Nacional de Investigaciones Cardiovasculares Carlos III CONSEJO SUPERIOR DE INVESTIGACIONES CIENTIFICAS Universidad Autónoma de Madrid. Application EP16382103. The sequence listing filed with the application follows.

SEQUENCE LISTING (26 sequences)

SEQ ID NO: 1 - DNA, 20 bp, Artificial Sequence
  Adamts1 primer
acactggcggttggcatcgt

SEQ ID NO: 2 - DNA, 20 bp, Artificial Sequence
  Adamts1 primer
gccagccctggtcaccttgc

SEQ ID NO: 3 - DNA, 21 bp, Artificial Sequence
  Nos2 primer
cagctgggctgtacaaacctt

SEQ ID NO: 4 - DNA, 21 bp, Artificial Sequence
  Nos2 primer
cattggaagtgaagcgtttcg

SEQ ID NO: 5 - DNA, 25 bp, Artificial Sequence
  Adamts1 mice primer
gccatcggggtcagcttttcaaatg

SEQ ID NO: 6 - DNA, 25 bp, Artificial Sequence
  Adamts1 mice primer
gggccagctcattcctcccactcat

SEQ ID NO: 7 - DNA, 25 bp, Artificial Sequence
  Adamts1 mice primer
ggttgtagtttcgcgctgagttttg

SEQ ID NO: 8 - DNA, 20 bp, Artificial Sequence
  Nos2-/- mice primer
acatgcagaatgagtaccgg

SEQ ID NO: 9 - DNA, 20 bp, Artificial Sequence
  Nos2-/- mice primer
tcaacatctcctggtggaac

SEQ ID NO: 10 - DNA, 20 bp, Artificial Sequence
  Nos2-/- mice primer
aatatgcgaagtggacctcg

SEQ ID NO: 11 - DNA, 21 bp, Artificial Sequence
  Fbn1C1039G/+ mice primer
ctcatcatttttggccagttg

SEQ ID NO: 12 - DNA, 20 bp, Artificial Sequence
  Fbn1C1039G/+ mice primer
gcacttgatgcacattcaca

SEQ ID NO: 13 - RNA, 29 nt, Artificial Sequence
  #siRNA27
ggaaagaatccgcagctttagtccactca

SEQ ID NO: 14 - RNA, 29 nt, Artificial Sequence
  #siRNA57
accgccagtgtcagtttacattcggagag

SEQ ID NO: 15 - RNA, 29 nt, Artificial Sequence
  #siRNA69
cttccgaatgtgcaaaggaagtgaagcca

SEQ ID NO: 16 - RNA, 19 nt, Artificial Sequence
  siCtl
gggtgaactcacgtcagaa

SEQ ID NO: 17 - DNA, 19 bp, Artificial Sequence
  Tgfß1 primer
cgccatctatgagaaaacc

SEQ ID NO: 18 - DNA, 17 bp, Artificial Sequence
  Tgfß1 primer
gtaacgccaggaattgt

SEQ ID NO: 19 - DNA, 18 bp, Artificial Sequence
  Ctgf primer
gtgccagaacgcacactg

SEQ ID NO: 20 - DNA, 18 bp, Artificial Sequence
  Ctgf primer
ccccggttacactccaaa

SEQ ID NO: 21 - DNA, 19 bp, Artificial Sequence
  Col1a1 primer
gctcctcttaggggccact

SEQ ID NO: 22 - DNA, 19 bp, Artificial Sequence
  Col1a1 primer
ccacgtctcaccattgggg

SEQ ID NO: 23 - DNA, 25 bp, Artificial Sequence
  Pai-1 primer
gccagatttatcatcaatgactggg

SEQ ID NO: 24 - DNA, 25 bp, Artificial Sequence
  Pai-1 primer
ggagaggtgcacatctttctcaaag

SEQ ID NO: 25 - DNA, 19 bp, Artificial Sequence
  Nos3 primer
gtttgtctgcggcgatgtc

SEQ ID NO: 26 - DNA, 17 bp, Artificial Sequence
  Nos3 primer
catgccgccctctgttg